European Patent Application EP 4 717 272 A1, published April 1, 2026. Title: Prdx3를 유효성분으로 포함하는 미토콘드리아 관련 질환 예방 또는 치료용 조성물 및 이의 용도. Applicant: 이화여자대학교 산학협력단. The sequence listing filed with the application follows.

SEQUENCE LISTING (12 sequences)

SEQ ID NO: 1 - DNA, 21 bp, synthetic construct
  source 1..21: mol_type = other DNA
aagccaagtccagctgcttcc

SEQ ID NO: 2 - DNA, 21 bp, synthetic construct
  source 1..21: mol_type = other DNA
gaagtgctttgtcatctaatt

SEQ ID NO: 3 - DNA, 21 bp, synthetic construct
  source 1..21: mol_type = other DNA
ggatacagtcaaagttgcagg

SEQ ID NO: 4 - DNA, 24 bp, synthetic construct
  source 1..24: mol_type = other DNA
caggaaatgtcaataagtgtctac

SEQ ID NO: 5 - DNA, 20 bp, synthetic construct
  source 1..20: mol_type = other DNA
ccagaggccacttgtgtagc

SEQ ID NO: 6 - DNA, 20 bp, synthetic construct
  source 1..20: mol_type = other DNA
cgaggaccagagcaaccttc

SEQ ID NO: 7 - DNA, 107 bp, synthetic construct
  source 1..107: mol_type = other DNA
atggcggcagctgcgggaaggttgctctggtcctcggttgctcgtcatgcaagtgctatttcccggagtatttctgcctcaacagttcttaggcctgttgcttctag

SEQ ID NO: 8 - DNA, 136 bp, synthetic construct
  source 1..136: mol_type = other DNA
aagaacctgtttgacagacatactgtggtctgcctctgcccaaggaaagtcagcctttagcaccagttcctctttccacacccctgctgtcacccagcacgcgccctattttaaaggtactgctgttgtcaatgga

SEQ ID NO: 9 - DNA, 143 bp, synthetic construct
  source 1..143: mol_type = other DNA
gagttcaaagagctgagtctcgacgactttaagggaaaatacttggtgcttttcttctaccctttggatttcacatttgtgtgtcctacagaaattgttgctttcagtgacaaagccaatgaatttcatgatgtaaactgtga

SEQ ID NO: 10 - DNA, 135 bp, synthetic construct
  source 1..135: mol_type = other DNA
agtagttgcagtttcagtggattcccacttcagtcatcttgcctggatcaacacaccaagaaagaatggtggtttgggccacatgaacatcacactgttgtcggatataactaagcagatatcccgagactacgg

SEQ ID NO: 11 - DNA, 104 bp, synthetic construct
  source 1..104: mol_type = other DNA
agtgctgttggaaagtgctggcattgcactcagaggtctcttcattattgaccctaatggtgtcgtcaagcacctgagtgtcaacgaccttccggtgggccgca

SEQ ID NO: 12 - DNA, 166 bp, synthetic construct
  source 1..166: mol_type = other DNA
gtgtggaagaaacactccgtttggtaaaggcgttccagtttgtggagacccatggagaagtctgcccagccaactggacaccagagtcccctacgatcaagccaagtccaacagcttccaaagagtactttgagaaggtccatcagtaggccatcctatgtctgca